European Patent Specification EP 4 059 947 B1, published January 10, 2024. Title: Novel protein variant and a method for producing L-valine using the same. Applicant: CJ CheilJedang Corporation. The sequence listing filed with the application follows.

SEQUENCE LISTING (11 sequences)

SEQ ID NO: 1 - protein, 422 aa, Artificial Sequence
  Protein variant
MRLNKRLPAALSGLLLSAALLAGCSTSGTAETTTTTVSSAAASTTTSTSSDSSSSSSSDSSTTAETISNTAEAAQAFLSTLSTEEQDAVLYDYDAEEKSTGWSNFPVTFVQRSGVNLTDLTEEQQAAALNVLKNLLNDDAYQMIEDIMASDQYLNDESNTTEDSLGQYYIAFFGDPSSDSDWSIQFGGHHIGINATFSDGAITFAPTHLGTQPSEWTNQDGETVAALSNMYETAFAFYDSLTEEQQAQLYQGKELDSMVCAPGSTCDYPTGTGLKGSDLTDEQKELLLDVIANWVGLADEETTETELDAIRETLDDTYINWSGATEYDTSTGDGIYFQISGPKVYIEFANQQGSAGADIDGVITAGWGHIHTIYRDPTNDYANSVTQEAASGMMGGGPGGNGGEMPSGDMPTGEMPSGAPSN

SEQ ID NO: 2 - DNA, 1269 bp, Artificial Sequence
  Protein variant coding gene
atgcgcctcaacaaacgactcccagcggcactctccggactgctgctctctgctgcccttcttgccggatgctccacttctggaaccgccgagaccacgacaacaaccgtttcatctgctgcggcatcaacaaccacttccacctcctccgattcctcttcctcctcttcctccgactcaagcaccaccgccgaaaccatctccaacaccgcggaagctgcccaagctttcttgtccaccctgtccaccgaagaacaagacgccgtactctacgactacgacgctgaagaaaagtccaccggctggtctaacttcccagtcaccttcgtgcagcgttccggcgtgaacctcaccgacctcactgaggaacagcaagcagctgccctcaacgtgctgaagaacctgctcaacgacgacgcctaccaaatgatcgaagacatcatggctagcgatcagtacctcaacgacgaaagcaacaccaccgaggattccctcggccagtactacatcgcattcttcggcgatccaagcagcgactccgactggtccatccaattcggcggacaccacatcggcatcaacgccaccttctccgacggtgccatcaccttcgccccaacccaccttggcacccagccttccgagtggaccaaccaggacggcgaaaccgttgcagcactaagcaacatgtacgaaaccgccttcgccttctacgacagcctcaccgaagagcagcaagcacagctctaccagggtaaagagttggattccatggtctgcgcaccgggcagcacctgcgactacccaaccggcaccggcttgaaaggctccgacctcaccgacgagcaaaaggaattgcttctcgacgtgatcgccaactgggttggtctagccgatgaggaaaccaccgaaactgaactcgatgccatccgcgaaaccctggatgacacctacatcaactggtccggagccaccgagtacgacacctccaccggcgacggcatctacttccagatcagtggcccaaaggtctacattgagttcgctaaccagcaaggttctgcaggtgccgacatcgacggtgtcatcaccgctggatggggccacattcacaccatctaccgcgacccaaccaatgattacgctaactccgtaactcaggaagcagccagcggaatgatgggcggcggccctggtggtaatggtggcgagatgcctagcggtgacatgcctactggtgaaatgccttctggcgctccatcaaactaa

SEQ ID NO: 3 - protein, 422 aa, Artificial Sequence
  Wild type protein
MRLNKRLPAALSGLLLSAALLAGCSTSGTAETTTTTVSSAAASTTTSTSSDSSSSSSSDSSTTAETISNTAEAAQAFLSTLSTEEQDAVLYDYDAEEKSTGWSNFPVTFVQRSGVNLTDLTEEQQAAALNVLKNLLNDDAYQMIEDIMASDQYLNDESNTTEDSLGQYYIAFFGDPSSDSDWSIQFGGHHIGINATFSDGAITFAPTHLGTQPSEWTNQDGETVAALSNMYETAFAFYDSLTEEQQAQLYQGEELDSMVCAPGSTCDYPTGTGLKGSDLTDEQKELLLDVIANWVGLADEETTETELDAIRETLDDTYINWSGATEYDTSTGDGIYFQISGPKVYIEFANQQGSAGADIDGVITAGWGHIHTIYRDPTNDYANSVTQEAASGMMGGGPGGNGGEMPSGDMPTGEMPSGAPSN

SEQ ID NO: 4 - DNA, 1269 bp, Artificial Sequence
  Wild type protein coding gene
atgcgcctcaacaaacgactcccagcggcactctccggactgctgctctctgctgcccttcttgccggatgctccacttctggaaccgccgagaccacgacaacaaccgtttcatctgctgcggcatcaacaaccacttccacctcctccgattcctcttcctcctcttcctccgactcaagcaccaccgccgaaaccatctccaacaccgcggaagctgcccaagctttcttgtccaccctgtccaccgaagaacaagacgccgtactctacgactacgacgctgaagaaaagtccaccggctggtctaacttcccagtcaccttcgtgcagcgttccggcgtgaacctcaccgacctcactgaggaacagcaagcagctgccctcaacgtgctgaagaacctgctcaacgacgacgcctaccaaatgatcgaagacatcatggctagcgatcagtacctcaacgacgaaagcaacaccaccgaggattccctcggccagtactacatcgcattcttcggcgatccaagcagcgactccgactggtccatccaattcggcggacaccacatcggcatcaacgccaccttctccgacggtgccatcaccttcgccccaacccaccttggcacccagccttccgagtggaccaaccaggacggcgaaaccgttgcagcactaagcaacatgtacgaaaccgccttcgccttctacgacagcctcaccgaagagcagcaagcacagctctaccagggtgaagagttggattccatggtctgcgcaccgggcagcacctgcgactacccaaccggcaccggcttgaaaggctccgacctcaccgacgagcaaaaggaattgcttctcgacgtgatcgccaactgggttggtctagccgatgaggaaaccaccgaaactgaactcgatgccatccgcgaaaccctggatgacacctacatcaactggtccggagccaccgagtacgacacctccaccggcgacggcatctacttccagatcagtggcccaaaggtctacattgagttcgctaaccagcaaggttctgcaggtgccgacatcgacggtgtcatcaccgctggatggggccacattcacaccatctaccgcgacccaaccaatgattacgctaactccgtaactcaggaagcagccagcggaatgatgggcggcggccctggtggtaatggtggcgagatgcctagcggtgacatgcctactggtgaaatgccttctggcgctccatcaaactaa

SEQ ID NO: 5 - DNA, 35 bp, Artificial Sequence
  NCgl2805_1F
tcgagctcggtacccaagacgccgtactctacgac

SEQ ID NO: 6 - DNA, 41 bp, Artificial Sequence
  NCgl2805_2R
accatggaatccaactctttaccctggtagagctgtgcttg

SEQ ID NO: 7 - DNA, 41 bp, Artificial Sequence
  NCgl2805_3F
caagcacagctctaccagggtaaagagttggattccatggt

SEQ ID NO: 8 - DNA, 35 bp, Artificial Sequence
  NCgl2805_4R
ctctagaggatccccagcgccagaaggcatttcac

SEQ ID NO: 9 - DNA, 20 bp, Artificial Sequence
  NCgl2805_5F
aagacgccgtactctacgac

SEQ ID NO: 10 - DNA, 20 bp, Artificial Sequence
  NCgl2805_6R
agcgccagaaggcatttcac

SEQ ID NO: 11 - DNA, 5803 bp, Artificial Sequence
  pDCM2
gttcgcttgctgtccataaaaccgcccagtctagctatcgccatgtaagcccactgcaagctacctgctttctctttgcgcttgcgttttcccttgtccagatagcccagtagctgacattcatccggggtcagcaccgtttctgcggactggctttctacgtgttccgcttcctttagcagcccttgcgccctgagtgcttgcggcagcgtgaagctagcttttatcgccattcgccattcaggctgcgcaactgttgggaagggcgatcggtgcgggcctcttcgctattacgccagctggcgaaagggggatgtgctgcaaggcgattaagttgggtaacgccagggttttcccagtcacgacgttgtaaaacgacggccagtgaattcgagctcggtacccggggatcctctagagtcgacctgcaggcatgcaagcttggcgtaatcatggtcatagctgtttcctgtgtgaaattgttatccgctcacaattccacacaacatacgagccggaagcataaagtgtaaagcctggggtgcctaatgagtgagctaactcacattaattgcgttgcgctcactgcccgctttccagtcgggaaacctgtcgtgccagctgcattaatgaatcggccaacgcgcggggagaggcggtttgcgtattgggcgctcttccgcttcctcgctcactgactcgctgcgctcggtcgttcggctgcggcgagcggtatcagctcactcaaaggcggtaatacggttatccacagaatcaggggataacgcaggaaagaacatgtgagcaaaaggccagcaaaaggccaggaaccgtaaaaaggccgcgttgctggcgtttttccataggctccgcccccctgacgagcatcacaaaaatcgacgctcaagtcagaggtggcgaaacccgacaggactataaagataccaggcgtttccccctggaagctccctcgtgcgctctcctgttccgaccctgccgcttaccggatacctgtccgcctttctcccttcgggaagcgtggcgctttctcaatgctcacgctgtaggtatctcagttcggtgtaggtcgttcgctccaagctgggctgtgtgcacgaaccccccgttcagcccgaccgctgcgccttatccggtaactatcgtcttgagtccaacccggtaagacacgacttatcgccactggcagcagccactggtaacaggattagcagagcgaggtatgtaggcggtgctacagagttcttgaagtggtggcctaactacggctacactagaaggacagtatttggtatctgcgctctgctgaagccagttaccttcggaaaaagagttggtagctcttgatccggcaaacaaaccaccgctggtagcggtggtttttttgtttgcaagcagcagattacgcgcagaaaaaaaggatctcaagaagatcctttgatcttttctacggggtctgacgctcagtggaacgaaaactcacgttaagggattttggtcatgagattatcaaaaaggatcttcacctagatccttttggggtgggcgaagaactccagcatgagatccccgcgctggaggatcatccagccctgatagaaacagaagccactggagcacctcaaaaacaccatcatacactaaatcagtaagttggcagcatcacccgacgcactttgcgccgaataaatacctgtgacggaagatcacttcgcagaataaataaatcctggtgtccctgttgataccgggaagccctgggccaacttttggcgaaaatgagacgttgatcggcacgtaagaggttccaactttcaccataatgaaataagatcactaccgggcgtattttttgagttatcgagattttcaggagctgatagaaacagaagccactggagcacctcaaaaacaccatcatacactaaatcagtaagttggcagcatcacccgacgcactttgcgccgaataaatacctgtgacggaagatcacttcgcagaataaataaatcctggtgtccctgttgataccgggaagccctgggccaacttttggcgaaaatgagacgttgatcggcacgtaagaggttccaactttcaccataatgaaataagatcactaccgggcgtattttttgagttatcgagattttcaggagctctttggcatcgtctctcgcctgtcccctcagttcagtaatttcctgcatttgcctgtttccagtcggtagatattccacaaaacagcagggaagcagcgcttttccgctgcataaccctgcttcggggtcattatagcgattttttcggtatatccatcctttttcgcacgatatacaggattttgccaaagggttcgtgtagactttccttggtgtatccaacggcgtcagccgggcaggataggtgaagtaggcccacccgcgagcgggtgttccttcttcactgtcccttattcgcacctggcggtgctcaacgggaatcctgctctgcgaggctggccggctaccgccggcgtaacagatgagggcaagcggatggctgatgaaaccaagccaaccaggaagggcagcccacctatcaaggtgtactgccttccagacgaacgaagagcgattgaggaaaaggcggcggcggccggcatgagcctgtcggcctacctgctggccgtcggccagggctacaaaatcacgggcgtcgtggactatgagcacgtccgcgagggcgtcccggaaaacgattccgaagcccaacctttcatagaaggcggcggtggaatcgaaatctcgtgatggcaggttgggcgtcgcttggtcggtcatttcgaaaaaggttaggaatacggttagccatttgcctgcttttatatagttcantatgggattcacctttatgttgataagaaataaaagaaaatgccaataggatatcggcattttcttttgcgtttttatttgttaactgttaattgtccttgttcaaggatgctgtctttgacaacagatgttttcttgcctttgatgttcagcaggaagctcggcgcaaacgttgattgtttgtctgcgtagaatcctctgtttgtcatatagcttgtaatcacgacattgtttcctttcgcttgaggtacagcgaagtgtgagtaagtaaaggttacatcgttaggcggatcaagatccatttttaacacaaggccagttttgttcagcggcttgtatgggccagttaaagaattagaaacataaccaagcatgtaaatatcgttagacgtaatgccgtcaatcgtcatttttgatccgcgggagtcagtgaacaggtaccatttgccgttcattttaaagacgttcgcgcgttcaatttcatctgttactgtgttagatgcaatcagcggtttcatcacttttttcagtgtgtaatcatcgtttagctcaatcataccgagagcgccgtttgctaactcagccgtgcgttttttatcgctttgcagaagtttttgactttcttgacggaagaatgatgtgcttttgccatagtatgctttgttaaataaagattcttcgccttggtagccatcttcagttccagtgtttgcttcaaatactaagtatttgtggcctttatcttctacgtagtgaggatctctcagcgtatggttgtcgcctgagctgtagttgccttcatcgatgaactgctgtacattttgatacgtttttccgtcaccgtcaaagattgatttataatcctctacaccgttgatgttcaaagagctgtctgatgctgatacgttaacttgtgcagttgtcagtgtttgtttgccgtaatgtttaccggagaaatcagtgtagaataaacggatttttccgtcagatgtaaatgtggctgaacctgaccattcttgtgtttggtcttttaggatagaatcatttgcatcgaatttgtcgctgtctttaaagacgcggccagcgtttttccagctgtcaatagaagtttcgccgactttttgatagaacatgtaaatcgatgtgtcatccgcatttttaggatctccggctaatgcaaagacgatgtggtagccgtgatagtttgcgacagtgccgtcagcgttttgtaatggccagctgtcccaaacgtccaggccttttgcagaagagatatttttaattgtggacgaatcaaattcagaaacttgatatttttcatttttttgctgttcagggatttgcagcatatcatggcgtgtaatatgggaaatgccgtatgtttccttatatggcttttggttcgtttctttcgcaaacgcttgagttgcgcctcctgccagcagtgcggtagtaaaggttaatactgttgcttgttttgcaaactttttgatgttcatcgttcatgtctccttttttatgtactgtgttagcggtctgcttcttccagccctcctgtttgaagatggcaagttagttacgcacaataaaaaaagacctaaaatatgtaaggggtgacgccaaagtatacactttgccctttacacattttaggtcttgcctgctttatcagtaacaaacccgcgcgatttacttttcgacctcattctattagactctcgtttggattgcaactggtctattttcctcttttgtttgatagaaaatcataaaaggatttgcagactacgggcctaaagaactaaaaaatctatctgtttcttttcattctctgtattttttatagtttctgttgcatgggcataaagttgcctttttaatcacaattcagaaaatatcataatatctcatttcactaaataatagtgaacggcaggtatatgtgatgggttaaaaaggatcaccccagagtcccgctcagaagaactcgtcaagaaggcgatagaaggcgatgcgctgcgaatcgggagcggcgataccgtaaagcacgaggaagcggtcagcccattcgccgccaagctcttcagcaatatcacgggtagccaacgctatgtcctgatagcggtccgccacacccagccggccacagtcgatgaatccagaaaagcggccattttccaccatgatattcggcaagcaggcatcgccatgggtcacgacgagatcctcgccgtcgggcatccgcgccttgagcctggcgaacagttcggctggcgcgagcccctgatgctcttcgtccagatcatcctgatcgacaagaccggcttccatccgagtacgtgctcgctcgatgcgatgtttcgcttggtggtcgaatgggcaggtagccggatcaagcgtatgcagccgccgcattgcatcagccatgatggatactttctcggcaggagcaaggtgagatgacaggagatcctgccccggcacttcgcccaatagcagccagtcccttcccgcttcagtgacaacgtcgagacagctgcgcaaggaacgcccgtcgtggccagccacgatagccgcgctgcctcgtcttggagttcattcagggcaccggacaggtcggtcttgacaaaaagaaccgggcgcccctgcgctgacagccggaacacggcggcatcagagcagccgattgtctgttgtgcccagtcatagccgaatagcctctccacccaagcggccggagaacctgcgtgcaatccatcttgttcaatcatgcgaaacgatcctcatcctgtctcttgatcagatcttgatcccctgcgccatcagatccttggcggcaagaaagccatccagtttactttgcagggcttcccaaccttaccagagggcgccccagctggcaattccg